European Patent Application EP 4 372 075 A1, published May 22, 2024. Title: Structure and use thereof. Applicant: 株式会社セルファイバ. Application JP. The sequence listing filed with the application follows.

SEQUENCE LISTING (20 sequences)

SEQ ID NO: 1 - DNA, 20 bp, synthetic construct
  source 1..20: mol_type = other DNA; note = Forward primer for NKX2.1
aggacaccatgaggaacagc

SEQ ID NO: 2 - DNA, 20 bp, synthetic construct
  source 1..20: mol_type = other DNA; note = Reverse primer for NKX2.1
gccatgttcttgctcacgtc

SEQ ID NO: 3 - DNA, 20 bp, synthetic construct
  source 1..20: mol_type = other DNA; note = Forward primer for SOX9
gaggaagtcggtgaagaacg

SEQ ID NO: 4 - DNA, 20 bp, synthetic construct
  source 1..20: mol_type = other DNA; note = Reverse primer for SOX9
atcgaaggtctcgatgttgg

SEQ ID NO: 5 - DNA, 20 bp, synthetic construct
  source 1..20: mol_type = other DNA; note = Forward primer for beta-actin
caatgtggccgaggactttg

SEQ ID NO: 6 - DNA, 22 bp, synthetic construct
  source 1..22: mol_type = other DNA; note = Reverse primer for beta-actin
cattctccttagagagaagtgg

SEQ ID NO: 7 - DNA, 20 bp, synthetic construct
  source 1..20: mol_type = other DNA; note = Forward primer for SFTPC
gcaaagaggtcctgatggag

SEQ ID NO: 8 - DNA, 20 bp, synthetic construct
  source 1..20: mol_type = other DNA; note = Reverse primer for SFTPC
tgtttctggctcatgtggag

SEQ ID NO: 9 - DNA, 22 bp, synthetic construct
  source 1..22: mol_type = other DNA; note = Forward primer for ABCA3
tctccttcagcttcatggtcag

SEQ ID NO: 10 - DNA, 21 bp, synthetic construct
  source 1..21: mol_type = other DNA; note = Reverse primer for ABCA3
tggctcagagtcatccagttg

SEQ ID NO: 11 - DNA, 21 bp, synthetic construct
  source 1..21: mol_type = other DNA; note = Forward primer for SFTPB
gagccgatgacctatgccaag

SEQ ID NO: 12 - DNA, 19 bp, synthetic construct
  source 1..19: mol_type = other DNA; note = Reverse primer for SFTPB
agcagcttcaaggggagga

SEQ ID NO: 13 - DNA, 20 bp, synthetic construct
  source 1..20: mol_type = other DNA; note = Forward primer for DCLAMP
accgatgtccaacttcaagc

SEQ ID NO: 14 - DNA, 20 bp, synthetic construct
  source 1..20: mol_type = other DNA; note = Reverse primer for DCLAMP
tgacaccttaggcggatttt

SEQ ID NO: 15 - DNA, 20 bp, synthetic construct
  source 1..20: mol_type = other DNA; note = Forward primer for SLC34A2
tcgccactgtcatcaagaag

SEQ ID NO: 16 - DNA, 22 bp, synthetic construct
  source 1..22: mol_type = other DNA; note = Reverse primer for SLC34A2
ctctgtacgatgaaggtcatgc

SEQ ID NO: 17 - DNA, 20 bp, synthetic construct
  source 1..20: mol_type = other DNA; note = Forward primer for FOXJ1
cctgtcggccatctacaagt

SEQ ID NO: 18 - DNA, 19 bp, synthetic construct
  source 1..19: mol_type = other DNA; note = Reverse primer for FOXJ1
agacaggttgtggcggatt

SEQ ID NO: 19 - DNA, 20 bp, synthetic construct
  source 1..20: mol_type = other DNA; note = Forward primer for SNTN
gctgcaaacccaatttagga

SEQ ID NO: 20 - DNA, 22 bp, synthetic construct
  source 1..22: mol_type = other DNA; note = Reverse primer for SNTN
tgctcatcaagttcagaaagga